European Patent Application EP 4 674 954 A1, published January 7, 2026. Title: TUMOR INFILTRATING LYMPHOCYTE EXPRESSING MEMBRANE-BOUND CYTOKINE. Applicant: Shanghai Juncell Therapeutics Co., Ltd. The sequence listing filed with the application follows.

SEQUENCE LISTING (50 sequences)

SEQ ID NO: 1 - protein, 24 aa, synthetic construct
MKRFLFLLLTISLLVMVQIQTGLS

SEQ ID NO: 2 - DNA, 72 bp, synthetic construct
  source 1..72: mol_type = other DNA
atgaagaggttcctgtttctgctgctgaccatcagcctgctggtcatggtgcagatccagaccggcctgtcc

SEQ ID NO: 3 - protein, 24 aa, synthetic construct
IYIWAPLAGTCGVLLLSLVITLYC

SEQ ID NO: 4 - DNA, 72 bp, synthetic construct
  source 1..72: mol_type = other DNA
atctacatctgggcgcccctggccgggacttgtggggtccttctcctgtcactggttatcaccctttactgc

SEQ ID NO: 5 - protein, 25 aa, synthetic construct
MFHVSFRYIFGLPPLILVLLPVASS

SEQ ID NO: 6 - DNA, 75 bp, synthetic construct
  source 1..75: mol_type = other DNA
atgttccatgtttcttttaggtatatctttggacttcctcccctgatccttgttctgttgccagtagcatcatct

SEQ ID NO: 7 - protein, 152 aa, synthetic construct
DCDIEGKDGKQYESVLMVSIDQLLDSMKEIGSNCLNNEFNFFKRHICDANKEGMFLFRAARKLRQFLKMNSTGDFDLHLLKVSEGTTILLNCTGQVKGRKPAALGEAQPTKSLEENKSLKEQKKLNDLCFLKRLLQEIKTCWNKILMGTKEH

SEQ ID NO: 8 - DNA, 456 bp, synthetic construct
  source 1..456: mol_type = other DNA
gattgtgatattgaaggtaaagatggcaaacaatatgagagtgttctaatggtcagcatcgatcaattattggacagcatgaaagaaattggtagcaattgcctgaataatgaatttaacttttttaaaagacatatctgtgatgctaataaggaaggtatgtttttattccgtgctgctcgcaagttgaggcaatttcttaaaatgaatagcactggtgattttgatctccacttattaaaagtttcagaaggcacaacaatactgttgaactgcactggccaggttaaaggaagaaaaccagctgccctgggtgaagcccaaccaacaaagagtttggaagaaaataaatctttaaaggaacagaaaaaactgaatgacttgtgtttcctaaagagactattacaagagataaaaacttgttggaataaaattttgatgggcactaaagaacac

SEQ ID NO: 9 - protein, 12 aa, synthetic construct
AEAAAKEAAAKA

SEQ ID NO: 10 - DNA, 36 bp, synthetic construct
  source 1..36: mol_type = other DNA
gccgaggccgccgccaaggaggccgccgccaaggcc

SEQ ID NO: 11 - protein, 9 aa, synthetic construct
RADAAPTVS

SEQ ID NO: 12 - DNA, 27 bp, synthetic construct
  source 1..27: mol_type = other DNA
agagctgatgccgctcctaccgtgagc

SEQ ID NO: 13 - protein, 9 aa, synthetic construct
GGGGSGGGG

SEQ ID NO: 14 - DNA, 27 bp, synthetic construct
  source 1..27: mol_type = other DNA
ggcggaggaggcagcggaggaggagga

SEQ ID NO: 15 - protein, 9 aa, synthetic construct
RTVAAPSVF

SEQ ID NO: 16 - DNA, 27 bp, synthetic construct
  source 1..27: mol_type = other DNA
aggaccgtggctgctcccagcgtgttc

SEQ ID NO: 17 - protein, 11 aa, synthetic construct
PSPLFPGPSKP

SEQ ID NO: 18 - DNA, 33 bp, synthetic construct
  source 1..33: mol_type = other DNA
ccttcccctctgttccctggaccatccaagccc

SEQ ID NO: 19 - protein, 55 aa, synthetic construct
FVPVFLPAKPTTTPAPRPPTPAPTIASQPLSLRPEACRPAAGGAVHTRGLDFACD

SEQ ID NO: 20 - DNA, 165 bp, synthetic construct
  source 1..165: mol_type = other DNA
ttcgtgccggtcttcctgccagcgaagcccaccacgacgccagcgccgcgaccaccaacaccggcgcccaccatcgcgtcgcagcccctgtccctgcgcccagaggcgtgccggccagcggcggggggcgcagtgcacacgagggggctggacttcgcctgtgat

SEQ ID NO: 21 - protein, 54 aa, synthetic construct
MLQMAGQCSQNEYFDSLLHACIPCQLRCSSNTPPLTCQRYCNASVTNSVKGTNA

SEQ ID NO: 22 - DNA, 162 bp, synthetic construct
  source 1..162: mol_type = other DNA
atgttgcagatggctgggcagtgctcccaaaatgaatattttgacagtttgttgcatgcttgcataccttgtcaacttcgatgttcttctaatactcctcctctaacatgtcagcgttattgtaatgcaagtgtgaccaattcagtgaaaggaacgaatgcg

SEQ ID NO: 23 - protein, 43 aa, synthetic construct
MLQMAGQCSQNEYFDSLLHACIPCQLRCSSNTPPLTCQRYCNA

SEQ ID NO: 24 - DNA, 129 bp, synthetic construct
  source 1..129: mol_type = other DNA
atgctgcagatggctggacagtgcagccagaacgagtacttcgacagcctgctgcacgcctgcatcccctgccagctgagatgcagcagcaacacccccccactgacctgtcagagatactgtaacgcc

SEQ ID NO: 25 - protein, 54 aa, synthetic construct
MLQMAGQCSQNEYFDSLLHACIPCDLRCSSNTPPLTCQRYCNASVTNSVKGTNA

SEQ ID NO: 26 - DNA, 162 bp, synthetic construct
  source 1..162: mol_type = other DNA
atgctgcagatggccggccagtgcagccagaacgagtacttcgactccctgctgcacgcctgcatcccttgcgacctgagatgtagctccaatacacctcctctgacatgccagagatactgcaacgccagcgtgaccaattccgtgaagggcaccaatgcc

SEQ ID NO: 27 - protein, 43 aa, synthetic construct
MLQMAGQCSQNEYFDSLLHACIPCDLRCSSNTPPLTCQRYCNA

SEQ ID NO: 28 - DNA, 129 bp, synthetic construct
  source 1..129: mol_type = other DNA
atgctgcagatggccggccagtgcagccagaacgagtacttcgactccctgctgcacgcctgcatcccttgcgacctgagatgtagctccaatacacctcctctgacatgccagagatactgcaacgcc

SEQ ID NO: 29 - protein, 37 aa, synthetic construct
GQNDTSQTSSPSASSNISGGIFLFFVANAIIHLFCFS

SEQ ID NO: 30 - DNA, 111 bp, synthetic construct
  source 1..111: mol_type = other DNA
ggccagaatgataccagccagacctcctccccttccgcttctagcaacatcagcggcggcatcttcctgttctttgtggccaacgccatcatccacctgttctgcttctcc

SEQ ID NO: 31 - protein, 279 aa, synthetic construct
MKRFLFLLLTISLLVMVQIQTGLSDCDIEGKDGKQYESVLMVSIDQLLDSMKEIGSNCLNNEFNFFKRHICDANKEGMFLFRAARKLRQFLKMNSTGDFDLHLLKVSEGTTILLNCTGQVKGRKPAALGEAQPTKSLEENKSLKEQKKLNDLCFLKRLLQEIKTCWNKILMGTKEHAEAAAKEAAAKAMLQMAGQCSQNEYFDSLLHACIPCQLRCSSNTPPLTCQRYCNASVTNSVKGTNAGQNDTSQTSSPSASSNISGGIFLFFVANAIIHLFCFS

SEQ ID NO: 32 - DNA, 840 bp, synthetic construct
  source 1..840: mol_type = other DNA
atgaagaggttcctgtttctgctgctgaccatcagcctgctggtcatggtgcagatccagaccggcctgtccgattgtgatattgaaggtaaagatggcaaacaatatgagagtgttctaatggtcagcatcgatcaattattggacagcatgaaagaaattggtagcaattgcctgaataatgaatttaacttttttaaaagacatatctgtgatgctaataaggaaggtatgtttttattccgtgctgctcgcaagttgaggcaatttcttaaaatgaatagcactggtgattttgatctccacttattaaaagtttcagaaggcacaacaatactgttgaactgcactggccaggttaaaggaagaaaaccagctgccctgggtgaagcccaaccaacaaagagtttggaagaaaataaatctttaaaggaacagaaaaaactgaatgacttgtgtttcctaaagagactattacaagagataaaaacttgttggaataaaattttgatgggcactaaagaacacgccgaggccgccgccaaggaggccgccgccaaggccatgttgcagatggctgggcagtgctcccaaaatgaatattttgacagtttgttgcatgcttgcataccttgtcaacttcgatgttcttctaatactcctcctctaacatgtcagcgttattgtaatgcaagtgtgaccaattcagtgaaaggaacgaatgcgggccagaatgataccagccagacctcctccccttccgcttctagcaacatcagcggcggcatcttcctgttctttgtggccaacgccatcatccacctgttctgcttctcctaa

SEQ ID NO: 33 - protein, 276 aa, synthetic construct
MKRFLFLLLTISLLVMVQIQTGLSDCDIEGKDGKQYESVLMVSIDQLLDSMKEIGSNCLNNEFNFFKRHICDANKEGMFLFRAARKLRQFLKMNSTGDFDLHLLKVSEGTTILLNCTGQVKGRKPAALGEAQPTKSLEENKSLKEQKKLNDLCFLKRLLQEIKTCWNKILMGTKEHRADAAPTVSMLQMAGQCSQNEYFDSLLHACIPCQLRCSSNTPPLTCQRYCNASVTNSVKGTNAGQNDTSQTSSPSASSNISGGIFLFFVANAIIHLFCFS

SEQ ID NO: 34 - DNA, 831 bp, synthetic construct
  source 1..831: mol_type = other DNA
atgaagaggttcctgtttctgctgctgaccatcagcctgctggtcatggtgcagatccagaccggcctgtccgattgtgatattgaaggtaaagatggcaaacaatatgagagtgttctaatggtcagcatcgatcaattattggacagcatgaaagaaattggtagcaattgcctgaataatgaatttaacttttttaaaagacatatctgtgatgctaataaggaaggtatgtttttattccgtgctgctcgcaagttgaggcaatttcttaaaatgaatagcactggtgattttgatctccacttattaaaagtttcagaaggcacaacaatactgttgaactgcactggccaggttaaaggaagaaaaccagctgccctgggtgaagcccaaccaacaaagagtttggaagaaaataaatctttaaaggaacagaaaaaactgaatgacttgtgtttcctaaagagactattacaagagataaaaacttgttggaataaaattttgatgggcactaaagaacacagagctgatgccgctcctaccgtgagcatgttgcagatggctgggcagtgctcccaaaatgaatattttgacagtttgttgcatgcttgcataccttgtcaacttcgatgttcttctaatactcctcctctaacatgtcagcgttattgtaatgcaagtgtgaccaattcagtgaaaggaacgaatgcgggccagaatgataccagccagacctcctccccttccgcttctagcaacatcagcggcggcatcttcctgttctttgtggccaacgccatcatccacctgttctgcttctcctaa

SEQ ID NO: 35 - protein, 276 aa, synthetic construct
MKRFLFLLLTISLLVMVQIQTGLSDCDIEGKDGKQYESVLMVSIDQLLDSMKEIGSNCLNNEFNFFKRHICDANKEGMFLFRAARKLRQFLKMNSTGDFDLHLLKVSEGTTILLNCTGQVKGRKPAALGEAQPTKSLEENKSLKEQKKLNDLCFLKRLLQEIKTCWNKILMGTKEHRTVAAPSVFMLQMAGQCSQNEYFDSLLHACIPCDLRCSSNTPPLTCQRYCNASVTNSVKGTNAGQNDTSQTSSPSASSNISGGIFLFFVANAIIHLFCFS

SEQ ID NO: 36 - DNA, 831 bp, synthetic construct
  source 1..831: mol_type = other DNA
atgaagaggttcctgtttctgctgctgaccatcagcctgctggtcatggtgcagatccagaccggcctgtccgattgtgatattgaaggtaaagatggcaaacaatatgagagtgttctaatggtcagcatcgatcaattattggacagcatgaaagaaattggtagcaattgcctgaataatgaatttaacttttttaaaagacatatctgtgatgctaataaggaaggtatgtttttattccgtgctgctcgcaagttgaggcaatttcttaaaatgaatagcactggtgattttgatctccacttattaaaagtttcagaaggcacaacaatactgttgaactgcactggccaggttaaaggaagaaaaccagctgccctgggtgaagcccaaccaacaaagagtttggaagaaaataaatctttaaaggaacagaaaaaactgaatgacttgtgtttcctaaagagactattacaagagataaaaacttgttggaataaaattttgatgggcactaaagaacacaggaccgtggctgctcccagcgtgttcatgctgcagatggccggccagtgcagccagaacgagtacttcgactccctgctgcacgcctgcatcccttgcgacctgagatgtagctccaatacacctcctctgacatgccagagatactgcaacgccagcgtgaccaattccgtgaagggcaccaatgccggccagaatgataccagccagacctcctccccttccgcttctagcaacatcagcggcggcatcttcctgttctttgtggccaacgccatcatccacctgttctgcttctcctaa

SEQ ID NO: 37 - protein, 322 aa, synthetic construct
MKRFLFLLLTISLLVMVQIQTGLSDCDIEGKDGKQYESVLMVSIDQLLDSMKEIGSNCLNNEFNFFKRHICDANKEGMFLFRAARKLRQFLKMNSTGDFDLHLLKVSEGTTILLNCTGQVKGRKPAALGEAQPTKSLEENKSLKEQKKLNDLCFLKRLLQEIKTCWNKILMGTKEHPSPLFPGPSKPMLQMAGQCSQNEYFDSLLHACIPCDLRCSSNTPPLTCQRYCNAFVPVFLPAKPTTTPAPRPPTPAPTIASQPLSLRPEACRPAAGGAVHTRGLDFACDGQNDTSQTSSPSASSNISGGIFLFFVANAIIHLFCFS

SEQ ID NO: 38 - DNA, 969 bp, synthetic construct
  source 1..969: mol_type = other DNA
atgaagaggttcctgtttctgctgctgaccatcagcctgctggtcatggtgcagatccagaccggcctgtccgattgtgatattgaaggtaaagatggcaaacaatatgagagtgttctaatggtcagcatcgatcaattattggacagcatgaaagaaattggtagcaattgcctgaataatgaatttaacttttttaaaagacatatctgtgatgctaataaggaaggtatgtttttattccgtgctgctcgcaagttgaggcaatttcttaaaatgaatagcactggtgattttgatctccacttattaaaagtttcagaaggcacaacaatactgttgaactgcactggccaggttaaaggaagaaaaccagctgccctgggtgaagcccaaccaacaaagagtttggaagaaaataaatctttaaaggaacagaaaaaactgaatgacttgtgtttcctaaagagactattacaagagataaaaacttgttggaataaaattttgatgggcactaaagaacacccttcccctctgttccctggaccatccaagcccatgctgcagatggccggccagtgcagccagaacgagtacttcgactccctgctgcacgcctgcatcccttgcgacctgagatgtagctccaatacacctcctctgacatgccagagatactgcaacgccttcgtgccggtcttcctgccagcgaagcccaccacgacgccagcgccgcgaccaccaacaccggcgcccaccatcgcgtcgcagcccctgtccctgcgcccagaggcgtgccggccagcggcggggggcgcagtgcacacgagggggctggacttcgcctgtgatggccagaatgataccagccagacctcctccccttccgcttctagcaacatcagcggcggcatcttcctgttctttgtggccaacgccatcatccacctgttctgcttctcctaa

SEQ ID NO: 39 - protein, 276 aa, synthetic construct
MKRFLFLLLTISLLVMVQIQTGLSDCDIEGKDGKQYESVLMVSIDQLLDSMKEIGSNCLNNEFNFFKRHICDANKEGMFLFRAARKLRQFLKMNSTGDFDLHLLKVSEGTTILLNCTGQVKGRKPAALGEAQPTKSLEENKSLKEQKKLNDLCFLKRLLQEIKTCWNKILMGTKEHMLQMAGQCSQNEYFDSLLHACIPCDLRCSSNTPPLTCQRYCNASVTNSVKGTNARTVAAPSVFGQNDTSQTSSPSASSNISGGIFLFFVANAIIHLFCFS

SEQ ID NO: 40 - DNA, 831 bp, synthetic construct
  source 1..831: mol_type = other DNA
atgaagaggttcctgtttctgctgctgaccatcagcctgctggtcatggtgcagatccagaccggcctgtccgattgtgatattgaaggtaaagatggcaaacaatatgagagtgttctaatggtcagcatcgatcaattattggacagcatgaaagaaattggtagcaattgcctgaataatgaatttaacttttttaaaagacatatctgtgatgctaataaggaaggtatgtttttattccgtgctgctcgcaagttgaggcaatttcttaaaatgaatagcactggtgattttgatctccacttattaaaagtttcagaaggcacaacaatactgttgaactgcactggccaggttaaaggaagaaaaccagctgccctgggtgaagcccaaccaacaaagagtttggaagaaaataaatctttaaaggaacagaaaaaactgaatgacttgtgtttcctaaagagactattacaagagataaaaacttgttggaataaaattttgatgggcactaaagaacacatgctgcagatggccggccagtgcagccagaacgagtacttcgactccctgctgcacgcctgcatcccttgcgacctgagatgtagctccaatacacctcctctgacatgccagagatactgcaacgccagcgtgaccaattccgtgaagggcaccaatgccaggaccgtggctgctcccagcgtgttcggccagaatgataccagccagacctcctccccttccgcttctagcaacatcagcggcggcatcttcctgttctttgtggccaacgccatcatccacctgttctgcttctcctaa

SEQ ID NO: 41 - protein, 276 aa, synthetic construct
MKRFLFLLLTISLLVMVQIQTGLSDCDIEGKDGKQYESVLMVSIDQLLDSMKEIGSNCLNNEFNFFKRHICDANKEGMFLFRAARKLRQFLKMNSTGDFDLHLLKVSEGTTILLNCTGQVKGRKPAALGEAQPTKSLEENKSLKEQKKLNDLCFLKRLLQEIKTCWNKILMGTKEHGGGGSGGGGMLQMAGQCSQNEYFDSLLHACIPCQLRCSSNTPPLTCQRYCNASVTNSVKGTNAGQNDTSQTSSPSASSNISGGIFLFFVANAIIHLFCFS

SEQ ID NO: 42 - DNA, 831 bp, synthetic construct
  source 1..831: mol_type = other DNA
atgaagaggttcctgtttctgctgctgaccatcagcctgctggtcatggtgcagatccagaccggcctgtccgattgtgatattgaaggtaaagatggcaaacaatatgagagtgttctaatggtcagcatcgatcaattattggacagcatgaaagaaattggtagcaattgcctgaataatgaatttaacttttttaaaagacatatctgtgatgctaataaggaaggtatgtttttattccgtgctgctcgcaagttgaggcaatttcttaaaatgaatagcactggtgattttgatctccacttattaaaagtttcagaaggcacaacaatactgttgaactgcactggccaggttaaaggaagaaaaccagctgccctgggtgaagcccaaccaacaaagagtttggaagaaaataaatctttaaaggaacagaaaaaactgaatgacttgtgtttcctaaagagactattacaagagataaaaacttgttggaataaaattttgatgggcactaaagaacacggcggaggaggcagcggaggaggaggaatgttgcagatggctgggcagtgctcccaaaatgaatattttgacagtttgttgcatgcttgcataccttgtcaacttcgatgttcttctaatactcctcctctaacatgtcagcgttattgtaatgcaagtgtgaccaattcagtgaaaggaacgaatgcgggccagaatgataccagccagacctcctccccttccgcttctagcaacatcagcggcggcatcttcctgttctttgtggccaacgccatcatccacctgttctgcttctcctaa

SEQ ID NO: 43 - protein, 263 aa, synthetic construct
MKRFLFLLLTISLLVMVQIQTGLSDCDIEGKDGKQYESVLMVSIDQLLDSMKEIGSNCLNNEFNFFKRHICDANKEGMFLFRAARKLRQFLKMNSTGDFDLHLLKVSEGTTILLNCTGQVKGRKPAALGEAQPTKSLEENKSLKEQKKLNDLCFLKRLLQEIKTCWNKILMGTKEHRADAAPTVSMLQMAGQCSQNEYFDSLLHACIPCQLRCSSNTPPLTCQRYCNASVTNSVKGTNAIYIWAPLAGTCGVLLLSLVITLYC

SEQ ID NO: 44 - DNA, 792 bp, synthetic construct
  source 1..792: mol_type = other DNA
atgaagaggttcctgtttctgctgctgaccatcagcctgctggtcatggtgcagatccagaccggcctgtccgattgtgatattgaaggtaaagatggcaaacaatatgagagtgttctaatggtcagcatcgatcaattattggacagcatgaaagaaattggtagcaattgcctgaataatgaatttaacttttttaaaagacatatctgtgatgctaataaggaaggtatgtttttattccgtgctgctcgcaagttgaggcaatttcttaaaatgaatagcactggtgattttgatctccacttattaaaagtttcagaaggcacaacaatactgttgaactgcactggccaggttaaaggaagaaaaccagctgccctgggtgaagcccaaccaacaaagagtttggaagaaaataaatctttaaaggaacagaaaaaactgaatgacttgtgtttcctaaagagactattacaagagataaaaacttgttggaataaaattttgatgggcactaaagaacacagagctgatgccgctcctaccgtgagcatgttgcagatggctgggcagtgctcccaaaatgaatattttgacagtttgttgcatgcttgcataccttgtcaacttcgatgttcttctaatactcctcctctaacatgtcagcgttattgtaatgcaagtgtgaccaattcagtgaaaggaacgaatgcgatctacatctgggcgcccctggccgggacttgtggggtccttctcctgtcactggttatcaccctttactgctaa

SEQ ID NO: 45 - protein, 266 aa, synthetic construct
MFHVSFRYIFGLPPLILVLLPVASSDCDIEGKDGKQYESVLMVSIDQLLDSMKEIGSNCLNNEFNFFKRHICDANKEGMFLFRAARKLRQFLKMNSTGDFDLHLLKVSEGTTILLNCTGQVKGRKPAALGEAQPTKSLEENKSLKEQKKLNDLCFLKRLLQEIKTCWNKILMGTKEHRADAAPTVSMLQMAGQCSQNEYFDSLLHACIPCQLRCSSNTPPLTCQRYCNAGQNDTSQTSSPSASSNISGGIFLFFVANAIIHLFCFS

SEQ ID NO: 46 - DNA, 801 bp, synthetic construct
  source 1..801: mol_type = other DNA
atgttccatgtttcttttaggtatatctttggacttcctcccctgatccttgttctgttgccagtagcatcatctgattgtgatattgaaggtaaagatggcaaacaatatgagagtgttctaatggtcagcatcgatcaattattggacagcatgaaagaaattggtagcaattgcctgaataatgaatttaacttttttaaaagacatatctgtgatgctaataaggaaggtatgtttttattccgtgctgctcgcaagttgaggcaatttcttaaaatgaatagcactggtgattttgatctccacttattaaaagtttcagaaggcacaacaatactgttgaactgcactggccaggttaaaggaagaaaaccagctgccctgggtgaagcccaaccaacaaagagtttggaagaaaataaatctttaaaggaacagaaaaaactgaatgacttgtgtttcctaaagagactattacaagagataaaaacttgttggaataaaattttgatgggcactaaagaacacagagctgatgccgctcctaccgtgagcatgctgcagatggctggacagtgcagccagaacgagtacttcgacagcctgctgcacgcctgcatcccctgccagctgagatgcagcagcaacacccccccactgacctgtcagagatactgtaacgccggccagaatgataccagccagacctcctccccttccgcttctagcaacatcagcggcggcatcttcctgttctttgtggccaacgccatcatccacctgttctgcttctcctaa

SEQ ID NO: 47 - protein, 267 aa, synthetic construct
MKRFLFLLLTISLLVMVQIQTGLSDCDIEGKDGKQYESVLMVSIDQLLDSMKEIGSNCLNNEFNFFKRHICDANKEGMFLFRAARKLRQFLKMNSTGDFDLHLLKVSEGTTILLNCTGQVKGRKPAALGEAQPTKSLEENKSLKEQKKLNDLCFLKRLLQEIKTCWNKILMGTKEHPSPLFPGPSKPMLQMAGQCSQNEYFDSLLHACIPCDLRCSSNTPPLTCQRYCNAGQNDTSQTSSPSASSNISGGIFLFFVANAIIHLFCFS

SEQ ID NO: 48 - DNA, 804 bp, synthetic construct
  source 1..804: mol_type = other DNA
atgaagaggttcctgtttctgctgctgaccatcagcctgctggtcatggtgcagatccagaccggcctgtccgattgtgatattgaaggtaaagatggcaaacaatatgagagtgttctaatggtcagcatcgatcaattattggacagcatgaaagaaattggtagcaattgcctgaataatgaatttaacttttttaaaagacatatctgtgatgctaataaggaaggtatgtttttattccgtgctgctcgcaagttgaggcaatttcttaaaatgaatagcactggtgattttgatctccacttattaaaagtttcagaaggcacaacaatactgttgaactgcactggccaggttaaaggaagaaaaccagctgccctgggtgaagcccaaccaacaaagagtttggaagaaaataaatctttaaaggaacagaaaaaactgaatgacttgtgtttcctaaagagactattacaagagataaaaacttgttggaataaaattttgatgggcactaaagaacacccttcccctctgttccctggaccatccaagcccatgctgcagatggccggccagtgcagccagaacgagtacttcgactccctgctgcacgcctgcatcccttgcgacctgagatgtagctccaatacacctcctctgacatgccagagatactgcaacgccggccagaatgataccagccagacctcctccccttccgcttctagcaacatcagcggcggcatcttcctgttctttgtggccaacgccatcatccacctgttctgcttctcctaa

SEQ ID NO: 49 - protein, 295 aa, synthetic construct
MALPVTALLLPLALLLHAARPQVQLQESGAELARPGASVKMSCKASGYTFTRYTMHWVKQRPGQGLEWIGYINPSRGYTNYNQKFKDKATLTTDKSSSTAYMQLSSLTSEDSAVYYCARYYDDHYCLDYWGQGTTLTVSSGGGGSGGGGSGGGGSDIVLTQSPAIMSASPGEKVTMTCSASSSVSYMNWYQQKSGTSPKRWIYDTSKLASGVPAHFRGSGSGTSYSLTISGMEAEDAATYYCQQWSSNPFTFGSGTKLEINRRADAAPTVSIYIWAPLAGTCGVLLLSLVITLYC

SEQ ID NO: 50 - DNA, 888 bp, synthetic construct
  source 1..888: mol_type = other DNA
atggccttaccagtgaccgccttgctcctgccgctggccttgctgctccacgccgccaggccgcaggtgcagctgcaggagtctggggctgaactggcaagacctggggcctcagtgaagatgtcctgcaaggcttctggctacacctttactaggtacacgatgcactgggtaaaacagaggcctggacagggtctggaatggattggatacattaatcctagccgtggttatactaattacaatcagaagttcaaggacaaggccacattgactacagacaaatcctccagcacagcctacatgcaactgagcagcctgacatctgaggactctgcagtctattactgtgcaagatattatgatgatcattactgccttgactactggggccaaggcaccactctcacagtctcctcaggcggaggaggcagcggcggaggaggcagcggcggaggaggcagcgatatcgtgctcactcagtctccagcaatcatgtctgcatctccaggggagaaggtcaccatgacctgcagtgccagctcaagtgtaagttacatgaactggtaccagcagaagtcaggcacctcccccaaaagatggatttatgacacatccaaactggcttctggagtccctgctcacttcaggggcagtgggtctgggacctcttactctctcacaatcagcggcatggaggctgaagatgctgccacttattactgccagcagtggagtagtaacccattcacgttcggctcggggacaaagttggaaataaaccggagagctgatgccgctcctaccgtgagcatctacatctgggcgcccctggccgggacttgtggggtccttctcctgtcactggttatcaccctttactgctaa